European Patent Application EP 4 745 156 A1, published May 20, 2026. Title: 可结合白介素31的抗体或其抗原结合片段及其制备方法和应用. Applicant: 北京伟杰信生物科技有限公司. The sequence listing filed with the application follows.

SEQUENCE LISTING (113 sequences)

SEQ ID NO: 1 - protein, 5 aa, synthetic construct
NYYLY

SEQ ID NO: 2 - protein, 17 aa, synthetic construct
ELNPRNGGTNLNAKFKT

SEQ ID NO: 3 - protein, 13 aa, synthetic construct
GGTTVVVRDVMDF

SEQ ID NO: 4 - protein, 15 aa, synthetic construct
RASESVDSYGNSFMH

SEQ ID NO: 5 - protein, 7 aa, synthetic construct
RASNLES

SEQ ID NO: 6 - protein, 9 aa, synthetic construct
QQSNEDPYT

SEQ ID NO: 7 - protein, 5 aa, synthetic construct
SYAMS

SEQ ID NO: 8 - protein, 17 aa, synthetic construct
YISNGGDYIFYADTVKG

SEQ ID NO: 9 - protein, 14 aa, synthetic construct
RGHYNTSSYWYFDV

SEQ ID NO: 10 - protein, 11 aa, synthetic construct
KASENVGTYVS

SEQ ID NO: 11 - protein, 7 aa, synthetic construct
GASNRYT

SEQ ID NO: 12 - protein, 9 aa, synthetic construct
GQSYSYPPT

SEQ ID NO: 13 - protein, 5 aa, synthetic construct
DAWMD

SEQ ID NO: 14 - protein, 19 aa, synthetic construct
EIRSRAESHATYYAESVKG

SEQ ID NO: 15 - protein, 12 aa, synthetic construct
ASTMITTGWFAY

SEQ ID NO: 16 - protein, 11 aa, synthetic construct
RASQNISVYLH

SEQ ID NO: 17 - protein, 7 aa, synthetic construct
YVSQSIS

SEQ ID NO: 18 - protein, 9 aa, synthetic construct
QNGHSFPYT

SEQ ID NO: 19 - protein, 7 aa, synthetic construct
GYSFTNY

SEQ ID NO: 20 - protein, 6 aa, synthetic construct
NPRNGG

SEQ ID NO: 21 - protein, 7 aa, synthetic construct
GFTFSSY

SEQ ID NO: 22 - protein, 6 aa, synthetic construct
SNGGDY

SEQ ID NO: 23 - protein, 7 aa, synthetic construct
GFTFSDA

SEQ ID NO: 24 - protein, 8 aa, synthetic construct
RSRAESHA

SEQ ID NO: 25 - protein, 8 aa, synthetic construct
GYSFTNYY

SEQ ID NO: 26 - protein, 8 aa, synthetic construct
LNPRNGGT

SEQ ID NO: 27 - protein, 15 aa, synthetic construct
TRGGTTVVVRDVMDF

SEQ ID NO: 28 - protein, 10 aa, synthetic construct
ESVDSYGNSF

SEQ ID NO: 29 - skipped

SEQ ID NO: 30 - protein, 8 aa, synthetic construct
GFTFSSYA

SEQ ID NO: 31 - protein, 8 aa, synthetic construct
ISNGGDYI

SEQ ID NO: 32 - protein, 16 aa, synthetic construct
TRRGHYNTSSYWYFDV

SEQ ID NO: 33 - protein, 6 aa, synthetic construct
ENVGTY

SEQ ID NO: 34 - skipped

SEQ ID NO: 35 - protein, 8 aa, synthetic construct
GFTFSDAW

SEQ ID NO: 36 - protein, 10 aa, synthetic construct
IRSRAESHAT

SEQ ID NO: 37 - protein, 14 aa, synthetic construct
TPASTMITTGWFAY

SEQ ID NO: 38 - protein, 6 aa, synthetic construct
QNISVY

SEQ ID NO: 39 - skipped

SEQ ID NO: 40 - protein, 122 aa, synthetic construct
EVQLQQSGAELVRPGASVRLSCKASGYSFTNYYLYWVKQRPGQGLEWIGELNPRNGGTNLNAKFKTKATLTVDKSSNTAYMRLSSLTSEDSAVYYCTRGGTTVVVRDVMDFWGQGTSVTVSS

SEQ ID NO: 41 - protein, 122 aa, synthetic construct
EVQLVESGGDLVKPGGSLRLSCVASGYSFTNYYLYWVRQAPGKGLEWVGELNPRNGGTNLNAKFKTRFTISVDKAKNMAYLQMNSLRAEDTAVYYCTRGGTTVVVRDVMDFWGQGTLVTVSS

SEQ ID NO: 42 - protein, 122 aa, synthetic construct
EVQLVESGGDLVKPGGSLRLSCVASGYSFTNYYLYWVRQAPGKGLQWLGELNPRNGGTNLNAKFKTRFTISVDKAKNTAYLQMNSLRAEDTAVYYCTRGGTTVVVRDVMDFWGQGTLVTVSS

SEQ ID NO: 43 - protein, 122 aa, synthetic construct
EVQLVESGGDLVKPGGSLRLSCVASGYSFTNYYLYWVRQAPGKGLEWVAELNPRNGGTNLNAKFKTRFTISRDNAKNMAYLQMNSLRAEDTAVYYCTRGGTTVVVRDVMDFWGQGTLVTVSS

SEQ ID NO: 44 - protein, 111 aa, synthetic construct
DIELTQSPASLAVSLGQRATISCRASESVDSYGNSFMHWYQQKPGQPPKLLIYRASNLESGIPARFSGSGSRTDFTLTINPVEADDVATYYCQQSNEDPYTFGGGTKLEIK

SEQ ID NO: 45 - protein, 111 aa, synthetic construct
EIVLTQTPLSLAVTPGELATISCRASESVDSYGNSFMHWYLQKPGQTPRLLIYRASNLESGVSDRFSGSGSRTDFTLKISRVEAEDVGVYYCQQSNEDPYTFGQGTKLEIK

SEQ ID NO: 46 - protein, 111 aa, synthetic construct
DIVLTQTPLSLSVSPGEPASISCRASESVDSYGNSFMHWYRQKPGQSPQLLIYRASNLESGVPDRFSGSGSRTDFTLRISRVEADDAGVYYCQQSNEDPYTFGQGTKLEIK

SEQ ID NO: 47 - protein, 111 aa, synthetic construct
DIVMTQTPLSLSVSPGEPASISCRASESVDSYGNSFMHWYRQKPGQSPQLLIYRASNLESGVPDRFSGSGSGTDFTLRISRVEADDAGVYYCQQSNEDPYTFGQGTKLEIK

SEQ ID NO: 48 - protein, 123 aa, synthetic construct
EVKLVESGEGLVKPGGSLKLSCAASGFTFSSYAMSWVRQTPEKRLEWVAYISNGGDYIFYADTVKGRFTISRDNARNTLYLQMSSLKSEDTAMYYCTRRGHYNTSSYWYFDVWGTGTTVTVSS

SEQ ID NO: 49 - protein, 123 aa, synthetic construct
EVQLVESGGDLVKPGGSLRLSCVASGFTFSSYAMSWVRQAPGKGLQWVAYISNGGDYIFYADTVKGRFTISRDNARNTLYLQMNSLRSEDTAVYYCTRRGHYNTSSYWYFDVWGQGTLVTVSS

SEQ ID NO: 50 - protein, 123 aa, synthetic construct
EVQLVESGGDLVKPGGSLRLSCVASGFTFSSYAMSWIRQAPGKGLQWVAYISNGGDYIFYADTVKGRFTISRDNAKNTLYLQMNSLRAEDTAVYYCTRRGHYNTSSYWYFDVWGQGTLVTVSS

SEQ ID NO: 51 - protein, 123 aa, synthetic construct
EVQLVESGGDLVKPGGSLRLSCVASGFTFSSYAMSWVRQAPGKGLQWVARISNGGDYIFYADTVKGRFTISRDNAKNTLYLQMNSLRAEDTAMYYCTRRGHYNTSSYWYFDVWGQGTLVTVSS

SEQ ID NO: 52 - protein, 107 aa, synthetic construct
DIVMTQSPKSMSMSVGERVTLSCKASENVGTYVSWYQQKPEQSPKLLIYGASNRYTGVPDRFTGSGSATDFTLTISSVQAEDLADYHCGQSYSYPPTFGAGTKLELK

SEQ ID NO: 53 - protein, 107 aa, synthetic construct
EIVMTQSPASLSLSQEEKVTITCKASENVGTYVSWYQQKPGQAPKLLIYGASNRYTGVPSRFSGSGSGTDFTFTISSLEPEDVAVYYCGQSYSYPPTFGAGTKVELK

SEQ ID NO: 54 - protein, 107 aa, synthetic construct
EIVMTQSPASLSLSQEEKVTITCKASENVGTYVSWYQQKPGQAPKLLIYGASNRYTGVPSRFSGSGSATDFTLTISSVEPEDVAVYYCGQSYSYPPTFGAGTKVELK

SEQ ID NO: 55 - protein, 107 aa, synthetic construct
EIVMTQSPASLSLSQEEKVTITCKASENVGTYVSWYQQKPGQAPKLLIYGASNRYTGVPSRFSGSGSGTDFSFTISSLEPEDVAVYYCGQSYSYPPTFGAGTKVELK

SEQ ID NO: 56 - protein, 123 aa, synthetic construct
EVKLVESGGGLVQPGGSMKLSCAASGFTFSDAWMDWVRQSPERGLEWVAEIRSRAESHATYYAESVKGRFTISRDDSKGSVYLQMNSLGTEDTGIYYCTPASTMITTGWFAYWGQGTMVTVSS

SEQ ID NO: 57 - protein, 123 aa, synthetic construct
EVQLVESGGDLVKPGGSLRLSCVASGFTFSDAWMDWVRQAPGKGLQWLAEIRSRAESHATYYAESVKGRFTISRDDAKNTVYLQMNSLRAEDTAVYYCTPASTMITTGWFAYWGQGTLVTVSS

SEQ ID NO: 58 - protein, 123 aa, synthetic construct
EVQLVESGGDLVKPGGSLRLSCVASGFTFSDAWMDWVRQAPGKGLEWVAEIRSRAESHATYYAESVKGRFTISRDDAKNMVYLQMNSLRAEDTAVYYCTPASTMITTGWFAYWGQGTLVTVSS

SEQ ID NO: 59 - protein, 123 aa, synthetic construct
EVQLVESGGDLVKPGGSLRLSCVASGFTFSDAWMDWVRQAPGKGLQWVAEIRSRAESHATYYAESVKGRFTISRDDAKNTVYLQMNSLRAEDTAVYYCTPASTMITTGWFAYWGQGTLVTVSS

SEQ ID NO: 60 - protein, 107 aa, synthetic construct
NIVMTQSPAILSVTPGDRVSLSCRASQNISVYLHWYQQKSHDSPRVLIKYVSQSISGIPSRFSGSGSGSDFTLRINSVEPEDVGVYYCQNGHSFPYTFGGGTKLEIK

SEQ ID NO: 61 - protein, 107 aa, synthetic construct
EIVMTQTPLSLAVTPGELATISCRASQNISVYLHWYLQKPGQTPRVLIKYVSQSISGVSDRFSGSGSGSDFTLKISRVEAEDVGVYYCQNGHSFPYTFGQGTKLEIK

SEQ ID NO: 62 - protein, 107 aa, synthetic construct
DIVMTQTPLSLSVSPGETASISCRASQNISVYLHWYRQKPGQSPQVLIKYVSQSISGVPDRFSGSGSGSDFTLRISRVEADDTGVYYCQNGHSFPYTFGQGTKLEIK

SEQ ID NO: 63 - protein, 107 aa, synthetic construct
EIVMTQTPLSLSVSPGELATISCRASQNISVYLHWYQQKPGQAPKVLIKYVSQSISGVPSRFSGSGSGSDFTLTISSVEAEDVGVYYCQNGHSFPYTFGQGTKLEIK

SEQ ID NO: 64 - protein, 335 aa, synthetic construct
ASTTAPSVFPLAPSCGSTSGSTVALACLVSGYFPEPVTVSWNSGSLTSGVHTFPSVLQSSGLYSLSSMVTVPSSRWPSETFTCNVAHPASKTKVDKPVPKRENGRVPRPPDCPKCPAPEAAGAPSVFIFPPKPKDTLLIARTPEVTCVVVDLDPEDPEVQISWFVDGKQMQTAKTQPREEQFNGTYRVVSVLPIGHQDWLKGKQFTCKVNNKALPSPIERTISKARGQAHQPSVYVLPPSREELSKNTVSLTCLIKDFFPPDIDVEWQSNGQQEPESKYRTTPPQLDEDGSYFLYSKLSVDKSRWQRGDTFICAVMHEALHNHYTQESLSHSPGK

SEQ ID NO: 65 - protein, 110 aa, synthetic construct
RNDAQPAVYLFQPSPDQLHTGSASVVCLLNSFYPKDINVKWKVDGVIQDTGIQESVTEQDKDSTYSLSSTLTMSSTEYLSHELYSCEITHKSLPSTLIKSFQRSECQRVD

SEQ ID NO: 66 - protein, 457 aa, synthetic construct
EVQLQQSGAELVRPGASVRLSCKASGYSFTNYYLYWVKQRPGQGLEWIGELNPRNGGTNLNAKFKTKATLTVDKSSNTAYMRLSSLTSEDSAVYYCTRGGTTVVVRDVMDFWGQGTSVTVSSASTTAPSVFPLAPSCGSTSGSTVALACLVSGYFPEPVTVSWNSGSLTSGVHTFPSVLQSSGLYSLSSMVTVPSSRWPSETFTCNVAHPASKTKVDKPVPKRENGRVPRPPDCPKCPAPEAAGAPSVFIFPPKPKDTLLIARTPEVTCVVVDLDPEDPEVQISWFVDGKQMQTAKTQPREEQFNGTYRVVSVLPIGHQDWLKGKQFTCKVNNKALPSPIERTISKARGQAHQPSVYVLPPSREELSKNTVSLTCLIKDFFPPDIDVEWQSNGQQEPESKYRTTPPQLDEDGSYFLYSKLSVDKSRWQRGDTFICAVMHEALHNHYTQESLSHSPGK

SEQ ID NO: 67 - protein, 457 aa, synthetic construct
EVQLVESGGDLVKPGGSLRLSCVASGYSFTNYYLYWVRQAPGKGLEWVGELNPRNGGTNLNAKFKTRFTISVDKAKNMAYLQMNSLRAEDTAVYYCTRGGTTVVVRDVMDFWGQGTLVTVSSASTTAPSVFPLAPSCGSTSGSTVALACLVSGYFPEPVTVSWNSGSLTSGVHTFPSVLQSSGLYSLSSMVTVPSSRWPSETFTCNVAHPASKTKVDKPVPKRENGRVPRPPDCPKCPAPEAAGAPSVFIFPPKPKDTLLIARTPEVTCVVVDLDPEDPEVQISWFVDGKQMQTAKTQPREEQFNGTYRVVSVLPIGHQDWLKGKQFTCKVNNKALPSPIERTISKARGQAHQPSVYVLPPSREELSKNTVSLTCLIKDFFPPDIDVEWQSNGQQEPESKYRTTPPQLDEDGSYFLYSKLSVDKSRWQRGDTFICAVMHEALHNHYTQESLSHSPGK

SEQ ID NO: 68 - protein, 457 aa, synthetic construct
EVQLVESGGDLVKPGGSLRLSCVASGYSFTNYYLYWVRQAPGKGLQWLGELNPRNGGTNLNAKFKTRFTISVDKAKNTAYLQMNSLRAEDTAVYYCTRGGTTVVVRDVMDFWGQGTLVTVSSASTTAPSVFPLAPSCGSTSGSTVALACLVSGYFPEPVTVSWNSGSLTSGVHTFPSVLQSSGLYSLSSMVTVPSSRWPSETFTCNVAHPASKTKVDKPVPKRENGRVPRPPDCPKCPAPEAAGAPSVFIFPPKPKDTLLIARTPEVTCVVVDLDPEDPEVQISWFVDGKQMQTAKTQPREEQFNGTYRVVSVLPIGHQDWLKGKQFTCKVNNKALPSPIERTISKARGQAHQPSVYVLPPSREELSKNTVSLTCLIKDFFPPDIDVEWQSNGQQEPESKYRTTPPQLDEDGSYFLYSKLSVDKSRWQRGDTFICAVMHEALHNHYTQESLSHSPGK

SEQ ID NO: 69 - protein, 457 aa, synthetic construct
EVQLVESGGDLVKPGGSLRLSCVASGYSFTNYYLYWVRQAPGKGLEWVAELNPRNGGTNLNAKFKTRFTISRDNAKNMAYLQMNSLRAEDTAVYYCTRGGTTVVVRDVMDFWGQGTLVTVSSASTTAPSVFPLAPSCGSTSGSTVALACLVSGYFPEPVTVSWNSGSLTSGVHTFPSVLQSSGLYSLSSMVTVPSSRWPSETFTCNVAHPASKTKVDKPVPKRENGRVPRPPDCPKCPAPEAAGAPSVFIFPPKPKDTLLIARTPEVTCVVVDLDPEDPEVQISWFVDGKQMQTAKTQPREEQFNGTYRVVSVLPIGHQDWLKGKQFTCKVNNKALPSPIERTISKARGQAHQPSVYVLPPSREELSKNTVSLTCLIKDFFPPDIDVEWQSNGQQEPESKYRTTPPQLDEDGSYFLYSKLSVDKSRWQRGDTFICAVMHEALHNHYTQESLSHSPGK

SEQ ID NO: 70 - protein, 221 aa, synthetic construct
DIELTQSPASLAVSLGQRATISCRASESVDSYGNSFMHWYQQKPGQPPKLLIYRASNLESGIPARFSGSGSRTDFTLTINPVEADDVATYYCQQSNEDPYTFGGGTKLEIKRNDAQPAVYLFQPSPDQLHTGSASVVCLLNSFYPKDINVKWKVDGVIQDTGIQESVTEQDKDSTYSLSSTLTMSSTEYLSHELYSCEITHKSLPSTLIKSFQRSECQRVD

SEQ ID NO: 71 - protein, 221 aa, synthetic construct
EIVLTQTPLSLAVTPGELATISCRASESVDSYGNSFMHWYLQKPGQTPRLLIYRASNLESGVSDRFSGSGSRTDFTLKISRVEAEDVGVYYCQQSNEDPYTFGQGTKLEIKRNDAQPAVYLFQPSPDQLHTGSASVVCLLNSFYPKDINVKWKVDGVIQDTGIQESVTEQDKDSTYSLSSTLTMSSTEYLSHELYSCEITHKSLPSTLIKSFQRSECQRVD

SEQ ID NO: 72 - protein, 221 aa, synthetic construct
DIVLTQTPLSLSVSPGEPASISCRASESVDSYGNSFMHWYRQKPGQSPQLLIYRASNLESGVPDRFSGSGSRTDFTLRISRVEADDAGVYYCQQSNEDPYTFGQGTKLEIKRNDAQPAVYLFQPSPDQLHTGSASVVCLLNSFYPKDINVKWKVDGVIQDTGIQESVTEQDKDSTYSLSSTLTMSSTEYLSHELYSCEITHKSLPSTLIKSFQRSECQRVD

SEQ ID NO: 73 - protein, 221 aa, synthetic construct
DIVMTQTPLSLSVSPGEPASISCRASESVDSYGNSFMHWYRQKPGQSPQLLIYRASNLESGVPDRFSGSGSGTDFTLRISRVEADDAGVYYCQQSNEDPYTFGQGTKLEIKRNDAQPAVYLFQPSPDQLHTGSASVVCLLNSFYPKDINVKWKVDGVIQDTGIQESVTEQDKDSTYSLSSTLTMSSTEYLSHELYSCEITHKSLPSTLIKSFQRSECQRVD

SEQ ID NO: 74 - protein, 458 aa, synthetic construct
EVKLVESGEGLVKPGGSLKLSCAASGFTFSSYAMSWVRQTPEKRLEWVAYISNGGDYIFYADTVKGRFTISRDNARNTLYLQMSSLKSEDTAMYYCTRRGHYNTSSYWYFDVWGTGTTVTVSSASTTAPSVFPLAPSCGSTSGSTVALACLVSGYFPEPVTVSWNSGSLTSGVHTFPSVLQSSGLYSLSSMVTVPSSRWPSETFTCNVAHPASKTKVDKPVPKRENGRVPRPPDCPKCPAPEAAGAPSVFIFPPKPKDTLLIARTPEVTCVVVDLDPEDPEVQISWFVDGKQMQTAKTQPREEQFNGTYRVVSVLPIGHQDWLKGKQFTCKVNNKALPSPIERTISKARGQAHQPSVYVLPPSREELSKNTVSLTCLIKDFFPPDIDVEWQSNGQQEPESKYRTTPPQLDEDGSYFLYSKLSVDKSRWQRGDTFICAVMHEALHNHYTQESLSHSPGK

SEQ ID NO: 75 - protein, 458 aa, synthetic construct
EVQLVESGGDLVKPGGSLRLSCVASGFTFSSYAMSWVRQAPGKGLQWVAYISNGGDYIFYADTVKGRFTISRDNARNTLYLQMNSLRSEDTAVYYCTRRGHYNTSSYWYFDVWGQGTLVTVSSASTTAPSVFPLAPSCGSTSGSTVALACLVSGYFPEPVTVSWNSGSLTSGVHTFPSVLQSSGLYSLSSMVTVPSSRWPSETFTCNVAHPASKTKVDKPVPKRENGRVPRPPDCPKCPAPEAAGAPSVFIFPPKPKDTLLIARTPEVTCVVVDLDPEDPEVQISWFVDGKQMQTAKTQPREEQFNGTYRVVSVLPIGHQDWLKGKQFTCKVNNKALPSPIERTISKARGQAHQPSVYVLPPSREELSKNTVSLTCLIKDFFPPDIDVEWQSNGQQEPESKYRTTPPQLDEDGSYFLYSKLSVDKSRWQRGDTFICAVMHEALHNHYTQESLSHSPGK

SEQ ID NO: 76 - protein, 458 aa, synthetic construct
EVQLVESGGDLVKPGGSLRLSCVASGFTFSSYAMSWIRQAPGKGLQWVAYISNGGDYIFYADTVKGRFTISRDNAKNTLYLQMNSLRAEDTAVYYCTRRGHYNTSSYWYFDVWGQGTLVTVSSASTTAPSVFPLAPSCGSTSGSTVALACLVSGYFPEPVTVSWNSGSLTSGVHTFPSVLQSSGLYSLSSMVTVPSSRWPSETFTCNVAHPASKTKVDKPVPKRENGRVPRPPDCPKCPAPEAAGAPSVFIFPPKPKDTLLIARTPEVTCVVVDLDPEDPEVQISWFVDGKQMQTAKTQPREEQFNGTYRVVSVLPIGHQDWLKGKQFTCKVNNKALPSPIERTISKARGQAHQPSVYVLPPSREELSKNTVSLTCLIKDFFPPDIDVEWQSNGQQEPESKYRTTPPQLDEDGSYFLYSKLSVDKSRWQRGDTFICAVMHEALHNHYTQESLSHSPGK

SEQ ID NO: 77 - protein, 458 aa, synthetic construct
EVQLVESGGDLVKPGGSLRLSCVASGFTFSSYAMSWVRQAPGKGLQWVAYISNGGDYIFYADTVKGRFTISRDNAKNTLYLQMNSLRAEDTAVYYCTRRGHYNTSSYWYFDVWGQGTLVTVSSASTTAPSVFPLAPSCGSTSGSTVALACLVSGYFPEPVTVSWNSGSLTSGVHTFPSVLQSSGLYSLSSMVTVPSSRWPSETFTCNVAHPASKTKVDKPVPKRENGRVPRPPDCPKCPAPEAAGAPSVFIFPPKPKDTLLIARTPEVTCVVVDLDPEDPEVQISWFVDGKQMQTAKTQPREEQFNGTYRVVSVLPIGHQDWLKGKQFTCKVNNKALPSPIERTISKARGQAHQPSVYVLPPSREELSKNTVSLTCLIKDFFPPDIDVEWQSNGQQEPESKYRTTPPQLDEDGSYFLYSKLSVDKSRWQRGDTFICAVMHEALHNHYTQESLSHSPGK

SEQ ID NO: 78 - protein, 217 aa, synthetic construct
DIVMTQSPKSMSMSVGERVTLSCKASENVGTYVSWYQQKPEQSPKLLIYGASNRYTGVPDRFTGSGSATDFTLTISSVQAEDLADYHCGQSYSYPPTFGAGTKLELKRNDAQPAVYLFQPSPDQLHTGSASVVCLLNSFYPKDINVKWKVDGVIQDTGIQESVTEQDKDSTYSLSSTLTMSSTEYLSHELYSCEITHKSLPSTLIKSFQRSECQRVD

SEQ ID NO: 79 - protein, 217 aa, synthetic construct
EIVMTQSPASLSLSQEEKVTITCKASENVGTYVSWYQQKPGQAPKLLIYGASNRYTGVPSRFSGSGSGTDFTFTISSLEPEDVAVYYCGQSYSYPPTFGAGTKVELKRNDAQPAVYLFQPSPDQLHTGSASVVCLLNSFYPKDINVKWKVDGVIQDTGIQESVTEQDKDSTYSLSSTLTMSSTEYLSHELYSCEITHKSLPSTLIKSFQRSECQRVD

SEQ ID NO: 80 - protein, 217 aa, synthetic construct
EIVMTQSPASLSLSQEEKVTITCKASENVGTYVSWYQQKPGQAPKLLIYGASNRYTGVPSRFSGSGSATDFTLTISSVEPEDVAVYYCGQSYSYPPTFGAGTKVELKRNDAQPAVYLFQPSPDQLHTGSASVVCLLNSFYPKDINVKWKVDGVIQDTGIQESVTEQDKDSTYSLSSTLTMSSTEYLSHELYSCEITHKSLPSTLIKSFQRSECQRVD

SEQ ID NO: 81 - protein, 217 aa, synthetic construct
EIVMTQSPASLSLSQEEKVTITCKASENVGTYVSWYQQKPGQAPKLLIYGASNRYTGVPSRFSGSGSGTDFSFTISSLEPEDVAVYYCGQSYSYPPTFGAGTKVELKRNDAQPAVYLFQPSPDQLHTGSASVVCLLNSFYPKDINVKWKVDGVIQDTGIQESVTEQDKDSTYSLSSTLTMSSTEYLSHELYSCEITHKSLPSTLIKSFQRSECQRVD

SEQ ID NO: 82 - protein, 458 aa, synthetic construct
EVKLVESGGGLVQPGGSMKLSCAASGFTFSDAWMDWVRQSPERGLEWVAEIRSRAESHATYYAESVKGRFTISRDDSKGSVYLQMNSLGTEDTGIYYCTPASTMITTGWFAYWGQGTMVTVSSASTTAPSVFPLAPSCGSTSGSTVALACLVSGYFPEPVTVSWNSGSLTSGVHTFPSVLQSSGLYSLSSMVTVPSSRWPSETFTCNVAHPASKTKVDKPVPKRENGRVPRPPDCPKCPAPEAAGAPSVFIFPPKPKDTLLIARTPEVTCVVVDLDPEDPEVQISWFVDGKQMQTAKTQPREEQFNGTYRVVSVLPIGHQDWLKGKQFTCKVNNKALPSPIERTISKARGQAHQPSVYVLPPSREELSKNTVSLTCLIKDFFPPDIDVEWQSNGQQEPESKYRTTPPQLDEDGSYFLYSKLSVDKSRWQRGDTFICAVMHEALHNHYTQESLSHSPGK

SEQ ID NO: 83 - protein, 458 aa, synthetic construct
EVQLVESGGDLVKPGGSLRLSCVASGFTFSDAWMDWVRQAPGKGLQWLAEIRSRAESHATYYAESVKGRFTISRDDAKNTVYLQMNSLRAEDTAVYYCTPASTMITTGWFAYWGQGTLVTVSSASTTAPSVFPLAPSCGSTSGSTVALACLVSGYFPEPVTVSWNSGSLTSGVHTFPSVLQSSGLYSLSSMVTVPSSRWPSETFTCNVAHPASKTKVDKPVPKRENGRVPRPPDCPKCPAPEAAGAPSVFIFPPKPKDTLLIARTPEVTCVVVDLDPEDPEVQISWFVDGKQMQTAKTQPREEQFNGTYRVVSVLPIGHQDWLKGKQFTCKVNNKALPSPIERTISKARGQAHQPSVYVLPPSREELSKNTVSLTCLIKDFFPPDIDVEWQSNGQQEPESKYRTTPPQLDEDGSYFLYSKLSVDKSRWQRGDTFICAVMHEALHNHYTQESLSHSPGK

SEQ ID NO: 84 - protein, 458 aa, synthetic construct
EVQLVESGGDLVKPGGSLRLSCVASGFTFSDAWMDWVRQAPGKGLEWVAEIRSRAESHATYYAESVKGRFTISRDDAKNMVYLQMNSLRAEDTAVYYCTPASTMITTGWFAYWGQGTLVTVSSASTTAPSVFPLAPSCGSTSGSTVALACLVSGYFPEPVTVSWNSGSLTSGVHTFPSVLQSSGLYSLSSMVTVPSSRWPSETFTCNVAHPASKTKVDKPVPKRENGRVPRPPDCPKCPAPEAAGAPSVFIFPPKPKDTLLIARTPEVTCVVVDLDPEDPEVQISWFVDGKQMQTAKTQPREEQFNGTYRVVSVLPIGHQDWLKGKQFTCKVNNKALPSPIERTISKARGQAHQPSVYVLPPSREELSKNTVSLTCLIKDFFPPDIDVEWQSNGQQEPESKYRTTPPQLDEDGSYFLYSKLSVDKSRWQRGDTFICAVMHEALHNHYTQESLSHSPGK

SEQ ID NO: 85 - protein, 458 aa, synthetic construct
EVQLVESGGDLVKPGGSLRLSCVASGFTFSDAWMDWVRQAPGKGLQWVAEIRSRAESHATYYAESVKGRFTISRDDAKNTVYLQMNSLRAEDTAVYYCTPASTMITTGWFAYWGQGTLVTVSSASTTAPSVFPLAPSCGSTSGSTVALACLVSGYFPEPVTVSWNSGSLTSGVHTFPSVLQSSGLYSLSSMVTVPSSRWPSETFTCNVAHPASKTKVDKPVPKRENGRVPRPPDCPKCPAPEAAGAPSVFIFPPKPKDTLLIARTPEVTCVVVDLDPEDPEVQISWFVDGKQMQTAKTQPREEQFNGTYRVVSVLPIGHQDWLKGKQFTCKVNNKALPSPIERTISKARGQAHQPSVYVLPPSREELSKNTVSLTCLIKDFFPPDIDVEWQSNGQQEPESKYRTTPPQLDEDGSYFLYSKLSVDKSRWQRGDTFICAVMHEALHNHYTQESLSHSPGK

SEQ ID NO: 86 - protein, 217 aa, synthetic construct
NIVMTQSPAILSVTPGDRVSLSCRASQNISVYLHWYQQKSHDSPRVLIKYVSQSISGIPSRFSGSGSGSDFTLRINSVEPEDVGVYYCQNGHSFPYTFGGGTKLEIKRNDAQPAVYLFQPSPDQLHTGSASVVCLLNSFYPKDINVKWKVDGVIQDTGIQESVTEQDKDSTYSLSSTLTMSSTEYLSHELYSCEITHKSLPSTLIKSFQRSECQRVD

SEQ ID NO: 87 - protein, 217 aa, synthetic construct
EIVMTQTPLSLAVTPGELATISCRASQNISVYLHWYLQKPGQTPRVLIKYVSQSISGVSDRFSGSGSGSDFTLKISRVEAEDVGVYYCQNGHSFPYTFGQGTKLEIKRNDAQPAVYLFQPSPDQLHTGSASVVCLLNSFYPKDINVKWKVDGVIQDTGIQESVTEQDKDSTYSLSSTLTMSSTEYLSHELYSCEITHKSLPSTLIKSFQRSECQRVD

SEQ ID NO: 88 - protein, 217 aa, synthetic construct
DIVMTQTPLSLSVSPGETASISCRASQNISVYLHWYRQKPGQSPQVLIKYVSQSISGVPDRFSGSGSGSDFTLRISRVEADDTGVYYCQNGHSFPYTFGQGTKLEIKRNDAQPAVYLFQPSPDQLHTGSASVVCLLNSFYPKDINVKWKVDGVIQDTGIQESVTEQDKDSTYSLSSTLTMSSTEYLSHELYSCEITHKSLPSTLIKSFQRSECQRVD

SEQ ID NO: 89 - protein, 217 aa, synthetic construct
EIVMTQTPLSLSVSPGELATISCRASQNISVYLHWYQQKPGQAPKVLIKYVSQSISGVPSRFSGSGSGSDFTLTISSVEAEDVGVYYCQNGHSFPYTFGQGTKLEIKRNDAQPAVYLFQPSPDQLHTGSASVVCLLNSFYPKDINVKWKVDGVIQDTGIQESVTEQDKDSTYSLSSTLTMSSTEYLSHELYSCEITHKSLPSTLIKSFQRSECQRVD

SEQ ID NO: 90 - DNA, 1371 bp, synthetic construct
  source 1..1371: mol_type = other DNA
gaggtgcagctgcagcagagcggcgctgagctggtcagacctggagcttctgtgcggctgtcttgcaaggccagtggctactcttttacaaactactacctgtactgggtcaagcagagacctggccagggcctggaatggatcggcgaactgaatcctcggaacggcggcaccaacctgaacgccaagttcaagaccaaggctacactgaccgtggataagtctagcaacacggcctacatgagactgtcttctctgacctccgaggactccgccgtgtactattgcaccagaggaggaaccaccgtggtcgtgcgggacgtgatggacttctggggccagggcacctctgtgacagtgtcctctgcctccaccaccgctcccagcgtgtttcccctggctcctagctgcggcagcacctccggatccaccgtggccctggcctgcctggtgtccggctacttcccagagcctgtcaccgtgtcctggaactccggctctctgacatcaggcgtgcatacctttccttctgtactgcagtcctccggactgtattccctctcctctatggtgactgtgccctcctccagatggccttccgaaaccttcacctgtaacgtggctcatcctgcttctaaaacaaaagtggacaagcccgtgcctaaaagagagaacggcagagtgccacggcctcctgactgccccaagtgccctgcccctgaggctgctggcgctcctagcgtgttcatcttcccccctaagcctaaggataccctgctgatcgccagaacccctgaagtgacctgtgtggttgtggacctggatcctgaggaccccgaagtgcagatctcttggttcgtggacggcaagcagatgcagaccgccaagacccagcctagggaggaacagttcaacggtacctacagagtggtgtccgtgctgccaatcggccaccaggactggctgaagggcaaacagttcacctgcaaggtgaacaacaaggccctgccctcacccatcgagcggaccatctccaaggctagaggccaggcccaccagccctccgtgtacgtgctgcctccttctcgcgaagagctcagcaagaacaccgtaagcctgacatgtctgatcaaagacttcttccctccagacattgatgtggaatggcagtctaatggccaacaagagcctgagtctaagtaccggacaacccctcctcagctggacgaggatggctcctacttcctgtactccaagctgtccgtggacaagtccagatggcagcggggcgacaccttcatctgcgccgtcatgcacgaggccctgcacaaccactacacccaagagtccctgagccactctcctggcaag

SEQ ID NO: 91 - DNA, 1371 bp, synthetic construct
  source 1..1371: mol_type = other DNA
gaagtgcagttggttgaaagcggaggagatttggttaagccaggggggtccttgcggctctcttgcgttgcatccggttacagttttaccaattattatctgtattgggtgcgccaagcacccggcaaaggattggagtgggtcggtgagctgaatcccaggaatggcggcaccaatctgaatgcaaaatttaagactcggtttactatctcagttgacaaggccaaaaacatggcgtacctccagatgaatagcctgcgcgcagaggatacagccgtttattactgtactagaggcggtactaccgtggtggtgagggacgtcatggacttttggggacagggcaccctggtgaccgtctcttccgcctccaccaccgctcccagcgtgtttcccctggctcctagctgcggcagcacctccggatccaccgtggccctggcctgcctggtgtccggctacttcccagagcctgtcaccgtgtcctggaactccggctctctgacatcaggcgtgcatacctttccttctgtactgcagtcctccggactgtattccctctcctctatggtgactgtgccctcctccagatggccttccgaaaccttcacctgtaacgtggctcatcctgcttctaaaacaaaagtggacaagcccgtgcctaaaagagagaacggcagagtgccacggcctcctgactgccccaagtgccctgcccctgaggctgctggcgctcctagcgtgttcatcttcccccctaagcctaaggataccctgctgatcgccagaacccctgaagtgacctgtgtggttgtggacctggatcctgaggaccccgaagtgcagatctcttggttcgtggacggcaagcagatgcagaccgccaagacccagcctagggaggaacagttcaacggtacctacagagtggtgtccgtgctgccaatcggccaccaggactggctgaagggcaaacagttcacctgcaaggtgaacaacaaggccctgccctcacccatcgagcggaccatctccaaggctagaggccaggcccaccagccctccgtgtacgtgctgcctccttctcgcgaagagctcagcaagaacaccgtaagcctgacatgtctgatcaaagacttcttccctccagacattgatgtggaatggcagtctaatggccaacaagagcctgagtctaagtaccggacaacccctcctcagctggacgaggatggctcctacttcctgtactccaagctgtccgtggacaagtccagatggcagcggggcgacaccttcatctgcgccgtcatgcacgaggccctgcacaaccactacacccaagagtccctgagccactctcctggcaag

SEQ ID NO: 92 - DNA, 1371 bp, synthetic construct
  source 1..1371: mol_type = other DNA
gaagtacaactggtggaatccgggggagatctcgtaaaaccaggagggagtctgcggctctcctgtgtggcttcaggctattctttcactaactattatctctattgggtgagacaggcccctggcaagggactgcaatggttgggggagctcaatccacggaacggcggaactaacctcaatgccaagtttaagaccaggtttacaatctcagtcgataaggccaagaacacggcgtatctgcagatgaatagcctgcgcgccgaggataccgctgtctactactgtaccagagggggaacgacagtcgtggtgagagacgtcatggatttttggggacaaggcactctcgtgaccgtgtcctctgcctccaccaccgctcccagcgtgtttcccctggctcctagctgcggcagcacctccggatccaccgtggccctggcctgcctggtgtccggctacttcccagagcctgtcaccgtgtcctggaactccggctctctgacatcaggcgtgcatacctttccttctgtactgcagtcctccggactgtattccctctcctctatggtgactgtgccctcctccagatggccttccgaaaccttcacctgtaacgtggctcatcctgcttctaaaacaaaagtggacaagcccgtgcctaaaagagagaacggcagagtgccacggcctcctgactgccccaagtgccctgcccctgaggctgctggcgctcctagcgtgttcatcttcccccctaagcctaaggataccctgctgatcgccagaacccctgaagtgacctgtgtggttgtggacctggatcctgaggaccccgaagtgcagatctcttggttcgtggacggcaagcagatgcagaccgccaagacccagcctagggaggaacagttcaacggtacctacagagtggtgtccgtgctgccaatcggccaccaggactggctgaagggcaaacagttcacctgcaaggtgaacaacaaggccctgccctcacccatcgagcggaccatctccaaggctagaggccaggcccaccagccctccgtgtacgtgctgcctccttctcgcgaagagctcagcaagaacaccgtaagcctgacatgtctgatcaaagacttcttccctccagacattgatgtggaatggcagtctaatggccaacaagagcctgagtctaagtaccggacaacccctcctcagctggacgaggatggctcctacttcctgtactccaagctgtccgtggacaagtccagatggcagcggggcgacaccttcatctgcgccgtcatgcacgaggccctgcacaaccactacacccaagagtccctgagccactctcctggcaag

SEQ ID NO: 93 - DNA, 1371 bp, synthetic construct
  source 1..1371: mol_type = other DNA
gaagtgcaactagtggaaagtggtggtgatctcgtgaagcctggaggctctctgcggctgtcttgtgtggcttctggctactcctttaccaactactatctgtactgggtcagacaggcccctggcaagggcctggaatgggtggccgagctgaacccccgcaacggcggaacaaacctgaatgctaagttcaaaacacggttcaccatctccagagataacgccaagaacatggcctacctgcagatgaactccctgagagctgaggacaccgccgtgtactactgcaccagaggcggcaccaccgttgtggtgcgggacgtgatggacttctggggccagggcaccctggtgaccgtgtccagcgcctccaccaccgctcccagcgtgtttcccctggctcctagctgcggcagcacctccggatccaccgtggccctggcctgcctggtgtccggctacttcccagagcctgtcaccgtgtcctggaactccggctctctgacatcaggcgtgcatacctttccttctgtactgcagtcctccggactgtattccctctcctctatggtgactgtgccctcctccagatggccttccgaaaccttcacctgtaacgtggctcatcctgcttctaaaacaaaagtggacaagcccgtgcctaaaagagagaacggcagagtgccacggcctcctgactgccccaagtgccctgcccctgaggctgctggcgctcctagcgtgttcatcttcccccctaagcctaaggataccctgctgatcgccagaacccctgaagtgacctgtgtggttgtggacctggatcctgaggaccccgaagtgcagatctcttggttcgtggacggcaagcagatgcagaccgccaagacccagcctagggaggaacagttcaacggtacctacagagtggtgtccgtgctgccaatcggccaccaggactggctgaagggcaaacagttcacctgcaaggtgaacaacaaggccctgccctcacccatcgagcggaccatctccaaggctagaggccaggcccaccagccctccgtgtacgtgctgcctccttctcgcgaagagctcagcaagaacaccgtaagcctgacatgtctgatcaaagacttcttccctccagacattgatgtggaatggcagtctaatggccaacaagagcctgagtctaagtaccggacaacccctcctcagctggacgaggatggctcctacttcctgtactccaagctgtccgtggacaagtccagatggcagcggggcgacaccttcatctgcgccgtcatgcacgaggccctgcacaaccactacacccaagagtccctgagccactctcctggcaag

SEQ ID NO: 94 - DNA, 663 bp, synthetic construct
  source 1..663: mol_type = other DNA
gacattgagctcacccagtctccagctagcctggctgtgtccctgggccagagagctaccatctcctgtagagcctctgaatctgtggactcctacggcaactccttcatgcactggtaccagcagaaacctggccaacctcctaagctgctgatctacagagcctccaacctggaatccggcatccctgccagattctctggctccggcagccggaccgacttcaccctgaccatcaatcctgtggaagctgacgacgttgccacctactactgccagcagtcgaacgaggatccctacaccttcggcggcggcaccaagctggaaatcaagcggaacgacgcccagcccgccgtgtacctgttccagccttctcctgaccagctgcacaccggctctgcttctgtcgtgtgcctgctgaactccttctaccccaaggatatcaacgtgaagtggaaggtggatggcgtgatccaggataccggaatccaagagtccgtgaccgagcaggacaaggactctacctattccctgtcttctacactgacaatgtccagcacagagtacctgtctcacgagctgtactcctgcgagatcacccataagtccctgccttccactctgatcaagtccttccagcggtccgagtgccagcgggtggac

SEQ ID NO: 95 - DNA, 663 bp, synthetic construct
  source 1..663: mol_type = other DNA
gagattgtgctgactcagacacctttgtctttggcagtgacccccggagagttggccacaatcagctgtagagccagtgaaagcgtggatagctacggaaacagtttcatgcactggtacttgcaaaagccagggcagacaccgcggctcctgatttatcgggcctcaaatctggagagcggcgttagcgataggttttccgggtccgggagtcgcaccgactttaccctgaaaatctccagggtcgaagcagaggatgtaggcgtatattactgccagcagagcaacgaggacccctacaccttcggtcagggcaccaaactcgagattaaacggaacgacgcccagcccgccgtgtacctgttccagccttctcctgaccagctgcacaccggctctgcttctgtcgtgtgcctgctgaactccttctaccccaaggatatcaacgtgaagtggaaggtggatggcgtgatccaggataccggaatccaagagtccgtgaccgagcaggacaaggactctacctattccctgtcttctacactgacaatgtccagcacagagtacctgtctcacgagctgtactcctgcgagatcacccataagtccctgccttccactctgatcaagtccttccagcggtccgagtgccagcgggtggac

SEQ ID NO: 96 - DNA, 663 bp, synthetic construct
  source 1..663: mol_type = other DNA
gacattgttctcacccagacacctctttcactgtctgtcagccctggggagcctgcctctatatcatgccgcgccagtgagtccgtggattcttacggtaattctttcatgcactggtacagacagaagcctggccaaagcccccagctgctgatctaccgggcttccaatctggagtccggggtccctgatagatttagcggatctggttcaaggacagatttcactctccggatttcacgagtggaggcagacgatgctggcgtgtactactgccagcagagcaatgaagatccctacactttcgggcagggcactaagctggagatcaagcggaacgacgcccagcccgccgtgtacctgttccagccttctcctgaccagctgcacaccggctctgcttctgtcgtgtgcctgctgaactccttctaccccaaggatatcaacgtgaagtggaaggtggatggcgtgatccaggataccggaatccaagagtccgtgaccgagcaggacaaggactctacctattccctgtcttctacactgacaatgtccagcacagagtacctgtctcacgagctgtactcctgcgagatcacccataagtccctgccttccactctgatcaagtccttccagcggtccgagtgccagcgggtggac

SEQ ID NO: 97 - DNA, 663 bp, synthetic construct
  source 1..663: mol_type = other DNA
gacattgtaatgacccagactcctctgtccctgagcgtttctcccggagagcctgcttcaattagctgcagagcatctgagtctgtggactcttacggcaactccttcatgcactggtaccggcaaaaacccggacagagcccacagctgctgatctacagggcctcaaacttggagagcggcgttcccgatagattcagcgggtctggaagcggaaccgattttaccctcagaatttccagagtggaggccgatgatgcgggcgtctactactgtcagcagagcaacgaggacccatatacatttggccaaggcactaagctggagatcaaacggaacgacgcccagcccgccgtgtacctgttccagccttctcctgaccagctgcacaccggctctgcttctgtcgtgtgcctgctgaactccttctaccccaaggatatcaacgtgaagtggaaggtggatggcgtgatccaggataccggaatccaagagtccgtgaccgagcaggacaaggactctacctattccctgtcttctacactgacaatgtccagcacagagtacctgtctcacgagctgtactcctgcgagatcacccataagtccctgccttccactctgatcaagtccttccagcggtccgagtgccagcgggtggac

SEQ ID NO: 98 - DNA, 1374 bp, synthetic construct
  source 1..1374: mol_type = other DNA
gaagtgaagctggtggagtctggggaaggcttagtgaagcctggagggtccctgaaactctcctgtgcagcctctggattcactttcagtagctatgccatgtcttgggttcgccagactccagagaagaggctggagtgggtcgcatacattagtaatggtggtgattacatcttctatgcagacactgtgaagggccgattcaccatctccagagacaatgccaggaacaccctgtacctgcaaatgagcagtctgaagtctgaggacacagccatgtattactgtacaagaaggggacattacaacactagtagttactggtacttcgatgtctggggcacagggaccacggtcaccgtctcctcagcctccaccaccgctcccagcgtgtttcccctggctcctagctgcggcagcacctccggatccaccgtggccctggcctgcctggtgtccggctacttcccagagcctgtcaccgtgtcctggaactccggctctctgacatcaggcgtgcatacctttccttctgtactgcagtcctccggactgtattccctctcctctatggtgactgtgccctcctccagatggccttccgaaaccttcacctgtaacgtggctcatcctgcttctaaaacaaaagtggacaagcccgtgcctaaaagagagaacggcagagtgccacggcctcctgactgccccaagtgccctgcccctgaggctgctggcgctcctagcgtgttcatcttcccccctaagcctaaggataccctgctgatcgccagaacccctgaagtgacctgtgtggttgtggacctggatcctgaggaccccgaagtgcagatctcttggttcgtggacggcaagcagatgcagaccgccaagacccagcctagggaggaacagttcaacggtacctacagagtggtgtccgtgctgccaatcggccaccaggactggctgaagggcaaacagttcacctgcaaggtgaacaacaaggccctgccctcacccatcgagcggaccatctccaaggctagaggccaggcccaccagccctccgtgtacgtgctgcctccttctcgcgaagagctcagcaagaacaccgtaagcctgacatgtctgatcaaagacttcttccctccagacattgatgtggaatggcagtctaatggccaacaagagcctgagtctaagtaccggacaacccctcctcagctggacgaggatggctcctacttcctgtactccaagctgtccgtggacaagtccagatggcagcggggcgacaccttcatctgcgccgtcatgcacgaggccctgcacaaccactacacccaagagtccctgagccactctcctggcaag

SEQ ID NO: 99 - DNA, 1374 bp, synthetic construct
  source 1..1374: mol_type = other DNA
gaagtccagcttgtagaatctggaggagaccttgtgaaaccaggcgggtcattgcggttgtcttgtgtggcgagtggcttcaccttcagcagttacgcaatgtcctgggtcagacaggcccccggaaaaggcttgcaatgggtggcttatatttctaatggtggggattatatcttttatgctgacacggtgaagggacgctttaccattagccgggacaatgccaggaacacactgtatctgcagatgaacagcctgcgcagcgaggacaccgccgtttactactgtacacgcagagggcactataacacctcttcctactggtacttcgacgtgtggggacagggcaccctggtgacagtgtcctctgcctccaccaccgctcccagcgtgtttcccctggctcctagctgcggcagcacctccggatccaccgtggccctggcctgcctggtgtccggctacttcccagagcctgtcaccgtgtcctggaactccggctctctgacatcaggcgtgcatacctttccttctgtactgcagtcctccggactgtattccctctcctctatggtgactgtgccctcctccagatggccttccgaaaccttcacctgtaacgtggctcatcctgcttctaaaacaaaagtggacaagcccgtgcctaaaagagagaacggcagagtgccacggcctcctgactgccccaagtgccctgcccctgaggctgctggcgctcctagcgtgttcatcttcccccctaagcctaaggataccctgctgatcgccagaacccctgaagtgacctgtgtggttgtggacctggatcctgaggaccccgaagtgcagatctcttggttcgtggacggcaagcagatgcagaccgccaagacccagcctagggaggaacagttcaacggtacctacagagtggtgtccgtgctgccaatcggccaccaggactggctgaagggcaaacagttcacctgcaaggtgaacaacaaggccctgccctcacccatcgagcggaccatctccaaggctagaggccaggcccaccagccctccgtgtacgtgctgcctccttctcgcgaagagctcagcaagaacaccgtaagcctgacatgtctgatcaaagacttcttccctccagacattgatgtggaatggcagtctaatggccaacaagagcctgagtctaagtaccggacaacccctcctcagctggacgaggatggctcctacttcctgtactccaagctgtccgtggacaagtccagatggcagcggggcgacaccttcatctgcgccgtcatgcacgaggccctgcacaaccactacacccaagagtccctgagccactctcctggcaag

SEQ ID NO: 100 - DNA, 1374 bp, synthetic construct
  source 1..1374: mol_type = other DNA
gaagttcagctggtggagtctggtggcgatttggtgaaaccaggtggttctctgcgcctgtcatgtgtagcttctggctttacatttagtagctacgcgatgagttggatccgacaggcacccggcaaagggcttcagtgggtggcatacatcagcaatggaggtgactatattttttatgctgatacagtcaaggggagattcacgatttccagggacaatgctaaaaataccctttacctgcagatgaacagcttgcgggccgaagacaccgccgtgtactattgtacccggagaggccactacaacacctcctcttattggtacttcgacgtgtggggccagggtaccctcgtgactgtgtccagcgcctccaccaccgctcccagcgtgtttcccctggctcctagctgcggcagcacctccggatccaccgtggccctggcctgcctggtgtccggctacttcccagagcctgtcaccgtgtcctggaactccggctctctgacatcaggcgtgcatacctttccttctgtactgcagtcctccggactgtattccctctcctctatggtgactgtgccctcctccagatggccttccgaaaccttcacctgtaacgtggctcatcctgcttctaaaacaaaagtggacaagcccgtgcctaaaagagagaacggcagagtgccacggcctcctgactgccccaagtgccctgcccctgaggctgctggcgctcctagcgtgttcatcttcccccctaagcctaaggataccctgctgatcgccagaacccctgaagtgacctgtgtggttgtggacctggatcctgaggaccccgaagtgcagatctcttggttcgtggacggcaagcagatgcagaccgccaagacccagcctagggaggaacagttcaacggtacctacagagtggtgtccgtgctgccaatcggccaccaggactggctgaagggcaaacagttcacctgcaaggtgaacaacaaggccctgccctcacccatcgagcggaccatctccaaggctagaggccaggcccaccagccctccgtgtacgtgctgcctccttctcgcgaagagctcagcaagaacaccgtaagcctgacatgtctgatcaaagacttcttccctccagacattgatgtggaatggcagtctaatggccaacaagagcctgagtctaagtaccggacaacccctcctcagctggacgaggatggctcctacttcctgtactccaagctgtccgtggacaagtccagatggcagcggggcgacaccttcatctgcgccgtcatgcacgaggccctgcacaaccactacacccaagagtccctgagccactctcctggcaag

SEQ ID NO: 101 - DNA, 1374 bp, synthetic construct
  source 1..1374: mol_type = other DNA
gaagtgcaactagtggaaagtggtggtgatctcgtgaagcccggaggatctctgcggctgtcttgtgtggcctctggcttcaccttcagctcttacgccatgtcctgggtgcggcaagctcctggcaagggcctgcagtgggtcgcttatatctccaacggcggcgactacatcttctacgctgatacagtgaaaggcagatttaccatctctcgggacaacgccaagaatacactgtacctgcagatgaactccctgagagccgaggacaccgccgtgtactactgcaccagaagaggccactacaacacctcctcctactggtacttcgacgtgtggggccagggcaccctggtgaccgtgtccagcgcctccaccaccgctcccagcgtgtttcccctggctcctagctgcggcagcacctccggatccaccgtggccctggcctgcctggtgtccggctacttcccagagcctgtcaccgtgtcctggaactccggctctctgacatcaggcgtgcatacctttccttctgtactgcagtcctccggactgtattccctctcctctatggtgactgtgccctcctccagatggccttccgaaaccttcacctgtaacgtggctcatcctgcttctaaaacaaaagtggacaagcccgtgcctaaaagagagaacggcagagtgccacggcctcctgactgccccaagtgccctgcccctgaggctgctggcgctcctagcgtgttcatcttcccccctaagcctaaggataccctgctgatcgccagaacccctgaagtgacctgtgtggttgtggacctggatcctgaggaccccgaagtgcagatctcttggttcgtggacggcaagcagatgcagaccgccaagacccagcctagggaggaacagttcaacggtacctacagagtggtgtccgtgctgccaatcggccaccaggactggctgaagggcaaacagttcacctgcaaggtgaacaacaaggccctgccctcacccatcgagcggaccatctccaaggctagaggccaggcccaccagccctccgtgtacgtgctgcctccttctcgcgaagagctcagcaagaacaccgtaagcctgacatgtctgatcaaagacttcttccctccagacattgatgtggaatggcagtctaatggccaacaagagcctgagtctaagtaccggacaacccctcctcagctggacgaggatggctcctacttcctgtactccaagctgtccgtggacaagtccagatggcagcggggcgacaccttcatctgcgccgtcatgcacgaggccctgcacaaccactacacccaagagtccctgagccactctcctggcaag

SEQ ID NO: 102 - DNA, 651 bp, synthetic construct
  source 1..651: mol_type = other DNA
gacattgtaatgacccaatctcccaaatccatgtccatgtcagtaggagagagggtcaccttgagctgcaaggccagtgagaatgtgggtacttatgtatcctggtatcaacagaaaccagagcagtctcctaaactgctgatatacggggcatccaaccggtacactggggtccccgatcgcttcacaggcagtggatctgcaacagatttcactctgaccatcagcagtgtgcaggctgaagaccttgcagattatcactgtggacagagttacagctatcctcccacgttcggtgctgggaccaagctggagctgaaacggaacgacgcccagcccgccgtgtacctgttccagccttctcctgaccagctgcacaccggctctgcttctgtcgtgtgcctgctgaactccttctaccccaaggatatcaacgtgaagtggaaggtggatggcgtgatccaggataccggaatccaagagtccgtgaccgagcaggacaaggactctacctattccctgtcttctacactgacaatgtccagcacagagtacctgtctcacgagctgtactcctgcgagatcacccataagtccctgccttccactctgatcaagtccttccagcggtccgagtgccagcgggtggac

SEQ ID NO: 103 - DNA, 651 bp, synthetic construct
  source 1..651: mol_type = other DNA
gagattgtgatgactcagtctccagcttccttgagcctgtcccaggaagaaaaggtgactatcacctgtaaagcctctgagaatgttggaacctacgtgtcctggtatcaacagaaaccagggcaggcacccaagttgctgatatacggcgcttccaacaggtacacaggcgtgccgtccaggttttccggctccggctcaggcacggacttcaccttcacaatttccagcctggaaccagaagatgtggccgtatattactgtgggcagtcttatagctacccaccaacatttggcgctggcactaaggtggagctgaaacggaacgacgcccagcccgccgtgtacctgttccagccttctcctgaccagctgcacaccggctctgcttctgtcgtgtgcctgctgaactccttctaccccaaggatatcaacgtgaagtggaaggtggatggcgtgatccaggataccggaatccaagagtccgtgaccgagcaggacaaggactctacctattccctgtcttctacactgacaatgtccagcacagagtacctgtctcacgagctgtactcctgcgagatcacccataagtccctgccttccactctgatcaagtccttccagcggtccgagtgccagcgggtggac

SEQ ID NO: 104 - DNA, 651 bp, synthetic construct
  source 1..651: mol_type = other DNA
gaaattgtcatgactcagagtccagccagtctgtcccttagccaggaagaaaaggtgactattacctgtaaggcctccgagaacgtggggacctatgtatcttggtaccaacagaagcctgggcaggcacccaaactgttgatatacggtgccagcaatcgatatactggagtgccatcacggttcagcggttctgggagcgctaccgacttcaccttgacaataagctccgtggaacccgaagacgtggcagtatactactgcggccagtcctactcatacccccctacttttggagccggtaccaaagtcgaattgaagcggaacgacgcccagcccgccgtgtacctgttccagccttctcctgaccagctgcacaccggctctgcttctgtcgtgtgcctgctgaactccttctaccccaaggatatcaacgtgaagtggaaggtggatggcgtgatccaggataccggaatccaagagtccgtgaccgagcaggacaaggactctacctattccctgtcttctacactgacaatgtccagcacagagtacctgtctcacgagctgtactcctgcgagatcacccataagtccctgccttccactctgatcaagtccttccagcggtccgagtgccagcgggtggac

SEQ ID NO: 105 - DNA, 651 bp, synthetic construct
  source 1..651: mol_type = other DNA
gaaatcgtgatgactcaaagtccagcaagtctgtccctgtctcaagaggaaaaagtgaccatcacctgcaaggcctctgagaacgtgggcacctacgtgtcctggtaccagcagaagcctggccaggctcctaagctgctgatctacggcgcctccaacagatacaccggcgtgccttctcggttctccggatctggcagcggaaccgacttcagcttcaccatctcctctctggaacccgaggatgtggccgtgtactactgtggccagtcctactcctatcctccaacatttggcgctggcaccaaggtcgagctgaagcggaacgacgcccagcccgccgtgtacctgttccagccttctcctgaccagctgcacaccggctctgcttctgtcgtgtgcctgctgaactccttctaccccaaggatatcaacgtgaagtggaaggtggatggcgtgatccaggataccggaatccaagagtccgtgaccgagcaggacaaggactctacctattccctgtcttctacactgacaatgtccagcacagagtacctgtctcacgagctgtactcctgcgagatcacccataagtccctgccttccactctgatcaagtccttccagcggtccgagtgccagcgggtggac

SEQ ID NO: 106 - DNA, 1374 bp, synthetic construct
  source 1..1374: mol_type = other DNA
gaggtgaaattggtagagtctggaggtgggcttgtacagccaggaggcagcatgaagttgtcatgcgccgcttcaggctttactttttcagacgcatggatggactgggttagacagtcaccagaaagaggcctggaatgggtcgccgagattcgcagtcgagcagagagccacgccacctattacgctgagtccgtcaagggccgcttcactatctctagggatgatagcaagggatctgtgtacctgcagatgaacagtctggggactgaggacaccggcatctattattgtacacctgccagtactatgatcactacgggctggtttgcctattggggacagggcactatggtgacagtgagctctgcctccaccaccgctcccagcgtgtttcccctggctcctagctgcggcagcacctccggatccaccgtggccctggcctgcctggtgtccggctacttcccagagcctgtcaccgtgtcctggaactccggctctctgacatcaggcgtgcatacctttccttctgtactgcagtcctccggactgtattccctctcctctatggtgactgtgccctcctccagatggccttccgaaaccttcacctgtaacgtggctcatcctgcttctaaaacaaaagtggacaagcccgtgcctaaaagagagaacggcagagtgccacggcctcctgactgccccaagtgccctgcccctgaggctgctggcgctcctagcgtgttcatcttcccccctaagcctaaggataccctgctgatcgccagaacccctgaagtgacctgtgtggttgtggacctggatcctgaggaccccgaagtgcagatctcttggttcgtggacggcaagcagatgcagaccgccaagacccagcctagggaggaacagttcaacggtacctacagagtggtgtccgtgctgccaatcggccaccaggactggctgaagggcaaacagttcacctgcaaggtgaacaacaaggccctgccctcacccatcgagcggaccatctccaaggctagaggccaggcccaccagccctccgtgtacgtgctgcctccttctcgcgaagagctcagcaagaacaccgtaagcctgacatgtctgatcaaagacttcttccctccagacattgatgtggaatggcagtctaatggccaacaagagcctgagtctaagtaccggacaacccctcctcagctggacgaggatggctcctacttcctgtactccaagctgtccgtggacaagtccagatggcagcggggcgacaccttcatctgcgccgtcatgcacgaggccctgcacaaccactacacccaagagtccctgagccactctcctggcaag

SEQ ID NO: 107 - DNA, 1374 bp, synthetic construct
  source 1..1374: mol_type = other DNA
gaggtgcagctggttgaaagtggcggagatctggttaaaccaggtggatccctgagacttagctgcgttgcaagtggcttcactttctccgatgcgtggatggattgggtgagacaggcccccgggaaaggactgcaatggcttgccgaaatacgcagcagagcagaatcacacgccacctactatgcagagtccgtcaagggcaggttcaccatttcacgcgatgacgccaaaaacacagtatatctgcagatgaacagcctcagggctgaggatacggccgtgtactactgtacaccggcctccactatgatcaccaccggctggtttgcctattggggacagggcactctggtgacggtcagcagcgcctccaccaccgctcccagcgtgtttcccctggctcctagctgcggcagcacctccggatccaccgtggccctggcctgcctggtgtccggctacttcccagagcctgtcaccgtgtcctggaactccggctctctgacatcaggcgtgcatacctttccttctgtactgcagtcctccggactgtattccctctcctctatggtgactgtgccctcctccagatggccttccgaaaccttcacctgtaacgtggctcatcctgcttctaaaacaaaagtggacaagcccgtgcctaaaagagagaacggcagagtgccacggcctcctgactgccccaagtgccctgcccctgaggctgctggcgctcctagcgtgttcatcttcccccctaagcctaaggataccctgctgatcgccagaacccctgaagtgacctgtgtggttgtggacctggatcctgaggaccccgaagtgcagatctcttggttcgtggacggcaagcagatgcagaccgccaagacccagcctagggaggaacagttcaacggtacctacagagtggtgtccgtgctgccaatcggccaccaggactggctgaagggcaaacagttcacctgcaaggtgaacaacaaggccctgccctcacccatcgagcggaccatctccaaggctagaggccaggcccaccagccctccgtgtacgtgctgcctccttctcgcgaagagctcagcaagaacaccgtaagcctgacatgtctgatcaaagacttcttccctccagacattgatgtggaatggcagtctaatggccaacaagagcctgagtctaagtaccggacaacccctcctcagctggacgaggatggctcctacttcctgtactccaagctgtccgtggacaagtccagatggcagcggggcgacaccttcatctgcgccgtcatgcacgaggccctgcacaaccactacacccaagagtccctgagccactctcctggcaag

SEQ ID NO: 108 - DNA, 1374 bp, synthetic construct
  source 1..1374: mol_type = other DNA
gaagttcagctggtagagtctggtggcgatctggttaagccaggaggcagcctgaggctttcttgtgtggccagcggattcacattctctgacgcctggatggactgggtgagacaagcccctggtaagggactggaatgggtggccgaaatcagatctagggccgaatcccatgcaacttattatgctgaatcagtcaaggggcgcttcacaatctccagagacgacgctaaaaatatggtgtacctgcaaatgaatagtcttcgggctgaggacaccgctgtgtactactgtacaccggcctccactatgattaccaccggatggtttgcctactgggggcagggaacattggtgacggtgtccagcgcctccaccaccgctcccagcgtgtttcccctggctcctagctgcggcagcacctccggatccaccgtggccctggcctgcctggtgtccggctacttcccagagcctgtcaccgtgtcctggaactccggctctctgacatcaggcgtgcatacctttccttctgtactgcagtcctccggactgtattccctctcctctatggtgactgtgccctcctccagatggccttccgaaaccttcacctgtaacgtggctcatcctgcttctaaaacaaaagtggacaagcccgtgcctaaaagagagaacggcagagtgccacggcctcctgactgccccaagtgccctgcccctgaggctgctggcgctcctagcgtgttcatcttcccccctaagcctaaggataccctgctgatcgccagaacccctgaagtgacctgtgtggttgtggacctggatcctgaggaccccgaagtgcagatctcttggttcgtggacggcaagcagatgcagaccgccaagacccagcctagggaggaacagttcaacggtacctacagagtggtgtccgtgctgccaatcggccaccaggactggctgaagggcaaacagttcacctgcaaggtgaacaacaaggccctgccctcacccatcgagcggaccatctccaaggctagaggccaggcccaccagccctccgtgtacgtgctgcctccttctcgcgaagagctcagcaagaacaccgtaagcctgacatgtctgatcaaagacttcttccctccagacattgatgtggaatggcagtctaatggccaacaagagcctgagtctaagtaccggacaacccctcctcagctggacgaggatggctcctacttcctgtactccaagctgtccgtggacaagtccagatggcagcggggcgacaccttcatctgcgccgtcatgcacgaggccctgcacaaccactacacccaagagtccctgagccactctcctggcaag

SEQ ID NO: 109 - DNA, 1374 bp, synthetic construct
  source 1..1374: mol_type = other DNA
gaggtgcaactcgtagaatccggtggcgatctggttaaaccaggaggttctcttagattgtcctgcgtggcctctgggttcaccttcagtgacgcttggatggactgggtgcggcaagctccaggaaagggattgcagtgggtggccgagatcagaagcagggcggagagccacgctacctactatgcagagtccgttaagggcagattcacaattagcagggatgacgcaaaaaatactgtctacctgcagatgaatagcctcagagcagaagataccgccgtgtattactgtacacctgcctccacgatgatcaccactggctggtttgcctactggggccaaggcactctcgtgacagtctcttccgcctccaccaccgctcccagcgtgtttcccctggctcctagctgcggcagcacctccggatccaccgtggccctggcctgcctggtgtccggctacttcccagagcctgtcaccgtgtcctggaactccggctctctgacatcaggcgtgcatacctttccttctgtactgcagtcctccggactgtattccctctcctctatggtgactgtgccctcctccagatggccttccgaaaccttcacctgtaacgtggctcatcctgcttctaaaacaaaagtggacaagcccgtgcctaaaagagagaacggcagagtgccacggcctcctgactgccccaagtgccctgcccctgaggctgctggcgctcctagcgtgttcatcttcccccctaagcctaaggataccctgctgatcgccagaacccctgaagtgacctgtgtggttgtggacctggatcctgaggaccccgaagtgcagatctcttggttcgtggacggcaagcagatgcagaccgccaagacccagcctagggaggaacagttcaacggtacctacagagtggtgtccgtgctgccaatcggccaccaggactggctgaagggcaaacagttcacctgcaaggtgaacaacaaggccctgccctcacccatcgagcggaccatctccaaggctagaggccaggcccaccagccctccgtgtacgtgctgcctccttctcgcgaagagctcagcaagaacaccgtaagcctgacatgtctgatcaaagacttcttccctccagacattgatgtggaatggcagtctaatggccaacaagagcctgagtctaagtaccggacaacccctcctcagctggacgaggatggctcctacttcctgtactccaagctgtccgtggacaagtccagatggcagcggggcgacaccttcatctgcgccgtcatgcacgaggccctgcacaaccactacacccaagagtccctgagccactctcctggcaag

SEQ ID NO: 110 - DNA, 651 bp, synthetic construct
  source 1..651: mol_type = other DNA
aacattgtgatgacccaatcccctgcaatcctgagtgtcactccaggggatagagtcagcctgagctgtcgggccagccaaaatatttctgtgtatttgcactggtaccagcaaaaaagccacgactcccccagggtgctcatcaaatacgtgagccagagtatcagcgggattccctcccgcttctccggatctgggagtggaagcgactttacactccgcataaattccgtcgagcctgaagatgtcggcgtgtactactgccagaacgggcacagctttccttacaccttcggggggggcacaaaattggaaatcaaacggaacgacgcccagcccgccgtgtacctgttccagccttctcctgaccagctgcacaccggctctgcttctgtcgtgtgcctgctgaactccttctaccccaaggatatcaacgtgaagtggaaggtggatggcgtgatccaggataccggaatccaagagtccgtgaccgagcaggacaaggactctacctattccctgtcttctacactgacaatgtccagcacagagtacctgtctcacgagctgtactcctgcgagatcacccataagtccctgccttccactctgatcaagtccttccagcggtccgagtgccagcgggtggac

SEQ ID NO: 111 - DNA, 651 bp, synthetic construct
  source 1..651: mol_type = other DNA
gagatagtgatgacacaaacgcccctgagtctcgccgtaacaccaggagagctggcgactatctcatgcagggccagccagaatatctccgtgtacctgcattggtacctgcagaaacctggccaaacacccagagtgctgattaagtatgtgtcccagtccatctccggggtctctgaccggttcagcggaagtggctctgggtccgactttaccttgaagatcagtagagtggaagcagaagacgtgggtgtctactactgccagaacgggcactcatttccatataccttcggacagggcacaaagctggaaatcaagcggaacgacgcccagcccgccgtgtacctgttccagccttctcctgaccagctgcacaccggctctgcttctgtcgtgtgcctgctgaactccttctaccccaaggatatcaacgtgaagtggaaggtggatggcgtgatccaggataccggaatccaagagtccgtgaccgagcaggacaaggactctacctattccctgtcttctacactgacaatgtccagcacagagtacctgtctcacgagctgtactcctgcgagatcacccataagtccctgccttccactctgatcaagtccttccagcggtccgagtgccagcgggtggac

SEQ ID NO: 112 - DNA, 651 bp, synthetic construct
  source 1..651: mol_type = other DNA
gacatcgtgatgacacaaacgcctctgtcactgagtgtgtcacccggtgaaacagccagtatttcatgtagggccagtcagaatatttccgtgtacctgcattggtacagacagaaacctgggcagagcccacaagtcctgatcaaatacgtctcacagtctattagtggggtccccgacagattctctggatcaggatctggtagcgacttcacactgagaatctcacgagttgaggccgacgacaccggcgtttactactgccagaatgggcactctttcccctacactttcggtcagggcaccaagttggagattaagcggaacgacgcccagcccgccgtgtacctgttccagccttctcctgaccagctgcacaccggctctgcttctgtcgtgtgcctgctgaactccttctaccccaaggatatcaacgtgaagtggaaggtggatggcgtgatccaggataccggaatccaagagtccgtgaccgagcaggacaaggactctacctattccctgtcttctacactgacaatgtccagcacagagtacctgtctcacgagctgtactcctgcgagatcacccataagtccctgccttccactctgatcaagtccttccagcggtccgagtgccagcgggtggac

SEQ ID NO: 113 - DNA, 651 bp, synthetic construct
  source 1..651: mol_type = other DNA
gagattgtaatgacacagacgcccctttctttgtccgtatctcctggcgagctcgctaccatcagttgcagggcatcccagaatatctcagtgtatctccactggtaccagcagaaaccaggacaggcacccaaagtcctgattaaatatgttagccagtctatctccggagtgccttctcggttcagcgggagcggcagcggctccgacttcaccctgactatctccagcgtcgaggctgaggacgtgggcgtgtactactgtcagaatgggcacagctttccatacaccttcggtcagggcacgaagctggagataaagcggaacgacgcccagcccgccgtgtacctgttccagccttctcctgaccagctgcacaccggctctgcttctgtcgtgtgcctgctgaactccttctaccccaaggatatcaacgtgaagtggaaggtggatggcgtgatccaggataccggaatccaagagtccgtgaccgagcaggacaaggactctacctattccctgtcttctacactgacaatgtccagcacagagtacctgtctcacgagctgtactcctgcgagatcacccataagtccctgccttccactctgatcaagtccttccagcggtccgagtgccagcgggtggac